European Patent Application EP 4 509 523 A1, published February 19, 2025. Title: Repaired KIR3DX1 and therapeutic uses thereof. Applicant: Deutsches Primatenzentrum GmbH (DPZ) Leibniz-Institut für Primatenforschung. Application EP. The sequence listing filed with the application follows.

SEQUENCE LISTING (62 sequences)

SEQ ID NO: 1 - protein, 99 aa, synthetic construct
GKYKKPSLSTQVDPMMRLGEKLTLFCSSEISFDQYHLFRHGVAHGQWLSGGQRHREAFQANFSVGRATPVPGGTYRCYGSFNDSPYEWSAPSDPLQLYT

SEQ ID NO: 2 - protein, 13 aa, unidentified
  SITE 4: note = A or R or N or D or C or Q or E or G or H or I or L or K or M or F or P or O or S or U or T or W or Y or V
  SITE 5: note = S or P
  SITE 13: note = A or R or N or D or C or Q or E or G or H or I or L or K or M or F or P or O or S or U or T or W or Y or V
  SITE 10: note = A or R or N or D or C or Q or E or G or H or I or L or K or M or F or P or O or S or U or T or W or Y or V
EWSXXSDPLXLYX

SEQ ID NO: 3 - protein, 13 aa, synthetic construct
EWSAPSDPLQLYT

SEQ ID NO: 4 - protein, 13 aa, Pan troglodytes
EWSAPSDPLQLYA

SEQ ID NO: 5 - protein, 93 aa, Homo sapiens
GAQDKFSLSAWPSPVVPLGGRVTLSCHSHLRFVIWTIFQTTGTRSHELHTGLSNNITISPVTPEHAGTYRCVGIYKHASKWSAESNSLKIIVT

SEQ ID NO: 6 - protein, 102 aa, Homo sapiens
GLFTKPSISAHPSSLVHAGARVSLRCHSELAFDEFILYKEGHIQHSQQLDQGMEAGIHYVEAVFSMGPVTPAHAGAYRCCGCFSHSRYEWSAPSDPLDIVIT

SEQ ID NO: 7 - protein, 325 aa, synthetic construct
GAQDKFSLSAWPSPVVPLGGRVTLSCHSHLRFVIWTIFQTTGTRSHELHTGLSNNITISPVTPEHAGTYRCVGIYKHASKWSAESNSLKIIVTGLFTKPSISAHPSSLVHAGARVSLRCHSELAFDEFILYKEGHIQHSQQLDQGMEAGIHYVEAVFSMGPVTPAHAGAYRCCGCFSHSRYEWSAPSDPLDIVITGKYKKPSLSTQVDPMMRLGEKLTLFCSSEISFDQYHLFRHGVAHGQWLSGGQRHREAFQANFSVGRATPVPGGTYRCYGSFNDSPYEWSAPSDPLQLYTTGNTKSTPLSFTESTPESDTPRPQGQSSNLH

SEQ ID NO: 8 - protein, 227 aa, Homo sapiens
DKTHTCPPCPAPELLGGPSVFLFPPKPKDTLMISRTPEVTCVVVDVSHEDPEVKFNWYVDGVEVHNAKTKPREEQYNSTYRVVSVLTVLHQDWLNGKEYKCKVSNKALPAPIEKTISKAKGQPREPQVYTLPPSREEMTKNQVSLTCLVKGFYPSDIAVEWESNGQPENNYKTTPPVLDSDGSFFLYSKLTVDKSRWQQGNVFSCSVMHEALHNHYTQKSLSLSPGK

SEQ ID NO: 9 - protein, 227 aa, Homo sapiens
ESKYGPPCPSCPAPEFLGGPSVFLFPPKPKDTLMISRTPEVTCVVVDVSQEDPEVQFNWYVDGVEVHNAKTKPREEQFNSTYRVVSVLTVLHQDWLNGKEYKCKVSNKGLPSSIEKTISKAKGQPREPQVYTLPPSQEEMTKNQVSLTCLVKGFYPSDIAVEWESNGQPENNYKTTPPVLDSDGSFFLYSRLTVDKSRWQEGNVFSCSVMHEALHNHYTQKSLSLSL

SEQ ID NO: 10 - protein, 34 aa, synthetic construct
TGNTKSTPLSFTESTPESDTPRPQGQSSNLHMLT

SEQ ID NO: 11 - protein, 23 aa, synthetic construct
GLSVAIISIGVCLSAFIGFWCYI

SEQ ID NO: 12 - protein, 85 aa, synthetic construct
KYHTTMANTEPTEGQRTDEEEPAAEETQEIIYAQLNHQALSQTGFPPASQCPHYLSEDPSIYITVHQAQAEARAAPSLWHKGHPR

SEQ ID NO: 13 - protein, 459 aa, synthetic construct
MAPKLITVLCLGFCLNQKICPHAGAQDKFSLSAWPSPVVPLGGRVTLSCHSHLRFVIWTIFQTTGTRSHELHTGLSNNITISPVTPEHAGTYRCVGIYKHASKWSAESNSLKIIVTGLFTKPSISAHPSSLVHAGARVSLRCHSELAFDEFILYKEGHIQHSQQLDQGMEAGIHYVEAVFSMGPVTPAHAGAYRCCGCFSHSRYEWSAPSDPLDIVITGKYKKPSLSTQVDPMMRLGEKLTLFCSSEISFDQYHLFRHGVAHGQWLSGGQRHREAFQANFSVGRATPVPGGTYRCYGSFNDSPYEWSAPSDPLQLYTTGNTKSTPLSFTESTPESDTPRPQGQSSNLHMLTGLSVAIISIGVCLSAFIGFWCYIKYHTTMANTEPTEGQRTDEEEPAAEETQEIIYAQLNHQALSQTGFPPASQCPHYLSEDPSIYITVHQAQAEARAAPSLWHKGHPR

SEQ ID NO: 14 - protein, 534 aa, synthetic construct
MAPKLITVLCLGFCLNQKICPHAGAQDKFSLSAWPSPVVPLGGRVTLSCHSHLRFVIWTIFQTTGTRSHELHTGLSNNITISPVTPEHAGTYRCVGIYKHASKWSAESNSLKIIVTGLFTKPSISAHPSSLVHAGARVSLRCHSELAFDEFILYKEGHIQHSQQLDQGMEAGIHYVEAVFSMGPVTPAHAGAYRCCGCFSHSRYEWSAPSDPLDIVITGKYKKPSLSTQVDPMMRLGEKLTLFCSSEISFDQYHLFRHGVAHGQWLSGGQRHREAFQANFSVGRATPVPGGTYRCYGSFNDSPYEWSAPSDPLQLYTTGNTKSTPLSFTESTPESDTPRPQGQSSNLHMLTLVVVGGVLACYSLLVTVAFIIFWVRSKRSRLLHSDYMNMTPRRPGPTRKHYQPYAPPRDFAAYRSASLRVKFSRSADAPAYQQGQNQLYNELNLGRREEYDVLDKRRGRDPEMGGKPQRRKNPQEGLYNELQKDKMAEAYSEIGMKGERRRGKGHDGLYQGLSTATKDTYDALHMQALPPRAS

SEQ ID NO: 15 - protein, 99 aa, Pan troglodytes
GKYKKPSLSTQVDPMMRLGEKLTLFCSSEISFDQYHLFRDGVAHGQWLSGGQRHRGAFQANFSVGRSMPVPGGTYRCYGSFNDSPYEWSAPSDPLQLYA

SEQ ID NO: 16 - protein, 99 aa, Gorilla gorilla
GKYKKPSLSTQVGPMMRLGEKLTLFCSSEISFDQYHLFRDGVAHGQWLSGGQRHRGAFQANFSVGPAMPVPGGTYRCYGSFNDSPYEWSAPSDPLQLYA

SEQ ID NO: 17 - protein, 99 aa, Pongo abelii
GKYKKPSLSTQVDPMIRLGEKLTFFCSSEISFDWYHLLRDGVAHGQWLSGGQRHSGAFQANFSVGPATPVPGGTYRCYGSFNDSPYEWSAPSDPLHLYV

SEQ ID NO: 18 - protein, 325 aa, Pan troglodytes
GAQDKFSLSAWPSPVVPLGGRVTLSCHSHLRFVIWTIFQTTGTRSHQLHTGLSNNITISPVTPGRAGTYRCVGIYKHTSKWSAESNSLKIIVTGLFTKPSISAHPSPLVHAGARVSLRCHSELAFDEFILYKEGHIQHSQQLDQGMEAGIHYVEAVFSVGPVTPAHAGAYRCCGCFSHSRYEWSAPSDPLDIVITGKYKKPSLSTQVDPMMRLGEKLTLFCSSEISFDQYHLFRDGVAHGQWLSGGQRHRGAFQANFSVGRSMPVPGGTYRCYGSFNDSPYEWSAPSDPLQLYATGNTKITPLSFTESTPESDTHRPQGQSSNLH

SEQ ID NO: 19 - protein, 325 aa, Gorilla gorilla
GAQDKFSLSAWPSPVVPLGGRVTLSCHSHLRFVIWTIFQTTGTRSHELHTGLSNNITISPVTPGHAGTYRCAGIYKHTSKWSAESNSLKIIVTGLFTKPSISAHPSSLVHAGARVSLRCHSELAFDEFILYKEGHIQHSQQLDQGMEAGIHYVEAVFSMGPITPAHAGAYRCCGCFSHSRYEWSAPSDSLDIVITGKYKKPSLSTQVGPMMRLGEKLTLFCSSEISFDQYHLFRDGVAHGQWLSGGQRHRGAFQANFSVGPAMPVPGGTYRCYGSFNDSPYEWSAPSDPLQLYATGNTKSTPLSFTESTPESDTHHPQGQSSNLH

SEQ ID NO: 20 - protein, 325 aa, Pongo abelii
GAQDKFSLSAWPSPVVPLGGRVTLSCHSRLRFVVWTIFQTTGTRSRELHIGLSNNITISPVTPGHAGTYKCVGIYKHTSKWSAESNSLKIIVTGLFTKPAISAHPSSLVHAGTRVSLRCHSELAFDEFILYKEGRIQYSQQLDQGMEAGIHYVEAVFSMGPVTPAHAGAYRCCGCFSHSSYEWSAPSDPLDIVITGKYKKPSLSTQVDPMIRLGEKLTFFCSSEISFDWYHLLRDGVAHGQWLSGGQRHSGAFQANFSVGPATPVPGGTYRCYGSFNDSPYEWSAPSDPLHLYVTGNTKSTPLSLMESTHESDTHHPQGQSSNLN

SEQ ID NO: 21 - DNA, 297 bp, synthetic construct
  source 1..297: mol_type = other DNA
ggaaaatacaaaaagccttctctctccacccaggtggaccccatgatgaggctgggagagaagttgaccctcttctgcagctctgaaatctcatttgaccagtaccatctgttcagacacggggttgctcatggacagtggctcagtggagggcagagacacagggaagcattccaggccaatttttctgtgggccgtgcaacgccagtccctggcgggacctatagatgctatggttccttcaatgactctccctatgagtggtcagcccccagtgacccgctgcaactttacacc

SEQ ID NO: 22 - DNA, 576 bp, synthetic construct
  source 1..576: mol_type = other DNA
ggtgctcaggacaagttctccctgtcagcctggccgagccctgtggttcccctaggaggacgtgtgactctctcctgtcattcccatcttcgatttgtcatatggacaatattccaaacaactgggacccgaagccatgagttgcacactggcctttccaacaacatcaccatcagccctgtgaccccagaacacgcagggacctacagatgtgttggaatttacaagcacgcctcaaagtggtcagctgagagcaactccctgaagatcatcgtcacaggaaaatacaaaaagccttctctctccacccaggtggaccccatgatgaggctgggagagaagttgaccctcttctgcagctctgaaatctcatttgaccagtaccatctgttcagacacggggttgctcatggacagtggctcagtggagggcagagacacagggaagcattccaggccaatttttctgtgggccgtgcaacgccagtccctggcgggacctatagatgctatggttccttcaatgactctccctatgagtggtcagcccccagtgacccgctgcaactttacacc

SEQ ID NO: 23 - DNA, 603 bp, synthetic construct
  source 1..603: mol_type = other DNA
ggcttgttcacaaaaccctccatctcagcgcacccaagctccctggtgcatgcaggagccagggtgagcctgcgctgtcactcagaactggcctttgatgaatttatcttatacaaagaggggcacatacagcattcccagcagcttgaccaggggatggaggctgggatccattacgtcgaggctgtcttttccatgggtcctgtaacgcctgcccatgcaggagcctacagatgctgtggttgtttcagtcactcccgctatgagtggtcggctcccagtgaccccctggacattgtgatcacaggaaaatacaaaaagccttctctctccacccaggtggaccccatgatgaggctgggagagaagttgaccctcttctgcagctctgaaatctcatttgaccagtaccatctgttcagacacggggttgctcatggacagtggctcagtggagggcagagacacagggaagcattccaggccaatttttctgtgggccgtgcaacgccagtccctggcgggacctatagatgctatggttccttcaatgactctccctatgagtggtcagcccccagtgacccgctgcaactttacacc

SEQ ID NO: 24 - DNA, 882 bp, synthetic construct
  source 1..882: mol_type = other DNA
ggtgctcaggacaagttctccctgtcagcctggccgagccctgtggttcccctaggaggacgtgtgactctctcctgtcattcccatcttcgatttgtcatatggacaatattccaaacaactgggacccgaagccatgagttgcacactggcctttccaacaacatcaccatcagccctgtgaccccagaacacgcagggacctacagatgtgttggaatttacaagcacgcctcaaagtggtcagctgagagcaactccctgaagatcatcgtcacaggcttgttcacaaaaccctccatctcagcgcacccaagctccctggtgcatgcaggagccagggtgagcctgcgctgtcactcagaactggcctttgatgaatttatcttatacaaagaggggcacatacagcattcccagcagcttgaccaggggatggaggctgggatccattacgtcgaggctgtcttttccatgggtcctgtaacgcctgcccatgcaggagcctacagatgctgtggttgtttcagtcactcccgctatgagtggtcggctcccagtgaccccctggacattgtgatcacaggaaaatacaaaaagccttctctctccacccaggtggaccccatgatgaggctgggagagaagttgaccctcttctgcagctctgaaatctcatttgaccagtaccatctgttcagacacggggttgctcatggacagtggctcagtggagggcagagacacagggaagcattccaggccaacttttctgtgggccgtgcaacgccagtccctggcgggacctatagatgctatggttccttcaatgactctccctatgagtggtcagcccccagtgacccgctgcaactttacacc

SEQ ID NO: 25 - DNA, 981 bp, synthetic construct
  source 1..981: mol_type = other DNA
ggaaaatacaaaaagccttctctctccacccaggtggaccccatgatgaggctgggagagaagttgaccctcttctgcagctctgaaatctcatttgaccagtaccatctgttcagacacggggttgctcatggacagtggctcagtggagggcagagacacagggaagcattccaggccaatttttctgtgggccgtgcaacgccagtccctggcgggacctatagatgctatggttccttcaatgactctccctatgagtggtcagcccccagtgacccgctgcaactttacaccgacaaaactcacacatgcccaccgtgcccagcacctgaactcctggggggaccgtcagtcttcctcttccccccaaaacccaaggacaccctcatgatctcccggacccctgaggtcacatgcgtggtggtggacgtgagccacgaagaccctgaggtcaagttcaactggtacgtggacggcgtggaggtgcataatgccaagacaaagccgcgggaggagcagtacaacagcacgtaccgtgtggtcagcgtcctcaccgtcctgcaccaggactggctgaatggcaaggagtacaagtgcaaggtctccaacaaagccctcccagcccccatcgagaaaaccatctccaaagccaaagggcagccccgagaaccacaggtgtacaccctgcccccatcccgggaggagatgaccaagaaccaggtcagcctgacctgcctggtcaaaggcttctatcccagcgacatcgccgtggagtgggagagcaatgggcagccggagaacaactacaagaccacgcctcccgtgctggactccgacggctccttcttcctctacagcaagctcaccgtggacaagagcaggtggcagcaggggaacgtcttctcatgctccgtgatgcacgaggctctgcacaaccactacacgcagaagagcctctccctgtctccgggtaaatga

SEQ ID NO: 26 - DNA, 1260 bp, synthetic construct
  source 1..1260: mol_type = other DNA
ggtgctcaggacaagttctccctgtcagcctggccgagccctgtggttcccctaggaggacgtgtgactctctcctgtcattcccatcttcgatttgtcatatggacaatattccaaacaactgggacccgaagccatgagttgcacactggcctttccaacaacatcaccatcagccctgtgaccccagaacacgcagggacctacagatgtgttggaatttacaagcacgcctcaaagtggtcagctgagagcaactccctgaagatcatcgtcacaggaaaatacaaaaagccttctctctccacccaggtggaccccatgatgaggctgggagagaagttgaccctcttctgcagctctgaaatctcatttgaccagtaccatctgttcagacacggggttgctcatggacagtggctcagtggagggcagagacacagggaagcattccaggccaatttttctgtgggccgtgcaacgccagtccctggcgggacctatagatgctatggttccttcaatgactctccctatgagtggtcagcccccagtgacccgctgcaactttacaccgacaaaactcacacatgcccaccgtgcccagcacctgaactcctggggggaccgtcagtcttcctcttccccccaaaacccaaggacaccctcatgatctcccggacccctgaggtcacatgcgtggtggtggacgtgagccacgaagaccctgaggtcaagttcaactggtacgtggacggcgtggaggtgcataatgccaagacaaagccgcgggaggagcagtacaacagcacgtaccgtgtggtcagcgtcctcaccgtcctgcaccaggactggctgaatggcaaggagtacaagtgcaaggtctccaacaaagccctcccagcccccatcgagaaaaccatctccaaagccaaagggcagccccgagaaccacaggtgtacaccctgcccccatcccgggaggagatgaccaagaaccaggtcagcctgacctgcctggtcaaaggcttctatcccagcgacatcgccgtggagtgggagagcaatgggcagccggagaacaactacaagaccacgcctcccgtgctggactccgacggctccttcttcctctacagcaagctcaccgtggacaagagcaggtggcagcaggggaacgtcttctcatgctccgtgatgcacgaggctctgcacaaccactacacgcagaagagcctctccctgtctccgggtaaatga

SEQ ID NO: 27 - DNA, 1287 bp, synthetic construct
  source 1..1287: mol_type = other DNA
ggcttgttcacaaaaccctccatctcagcgcacccaagctccctggtgcatgcaggagccagggtgagcctgcgctgtcactcagaactggcctttgatgaatttatcttatacaaagaggggcacatacagcattcccagcagcttgaccaggggatggaggctgggatccattacgtcgaggctgtcttttccatgggtcctgtaacgcctgcccatgcaggagcctacagatgctgtggttgtttcagtcactcccgctatgagtggtcggctcccagtgaccccctggacattgtgatcacaggaaaatacaaaaagccttctctctccacccaggtggaccccatgatgaggctgggagagaagttgaccctcttctgcagctctgaaatctcatttgaccagtaccatctgttcagacacggggttgctcatggacagtggctcagtggagggcagagacacagggaagcattccaggccaatttttctgtgggccgtgcaacgccagtccctggcgggacctatagatgctatggttccttcaatgactctccctatgagtggtcagcccccagtgacccgctgcaactttacaccgacaaaactcacacatgcccaccgtgcccagcacctgaactcctggggggaccgtcagtcttcctcttccccccaaaacccaaggacaccctcatgatctcccggacccctgaggtcacatgcgtggtggtggacgtgagccacgaagaccctgaggtcaagttcaactggtacgtggacggcgtggaggtgcataatgccaagacaaagccgcgggaggagcagtacaacagcacgtaccgtgtggtcagcgtcctcaccgtcctgcaccaggactggctgaatggcaaggagtacaagtgcaaggtctccaacaaagccctcccagcccccatcgagaaaaccatctccaaagccaaagggcagccccgagaaccacaggtgtacaccctgcccccatcccgggaggagatgaccaagaaccaggtcagcctgacctgcctggtcaaaggcttctatcccagcgacatcgccgtggagtgggagagcaatgggcagccggagaacaactacaagaccacgcctcccgtgctggactccgacggctccttcttcctctacagcaagctcaccgtggacaagagcaggtggcagcaggggaacgtcttctcatgctccgtgatgcacgaggctctgcacaaccactacacgcagaagagcctctccctgtctccgggtaaatga

SEQ ID NO: 28 - DNA, 1566 bp, synthetic construct
  source 1..1566: mol_type = other DNA
ggtgctcaggacaagttctccctgtcagcctggccgagccctgtggttcccctaggaggacgtgtgactctctcctgtcattcccatcttcgatttgtcatatggacaatattccaaacaactgggacccgaagccatgagttgcacactggcctttccaacaacatcaccatcagccctgtgaccccagaacacgcagggacctacagatgtgttggaatttacaagcacgcctcaaagtggtcagctgagagcaactccctgaagatcatcgtcacaggcttgttcacaaaaccctccatctcagcgcacccaagctccctggtgcatgcaggagccagggtgagcctgcgctgtcactcagaactggcctttgatgaatttatcttatacaaagaggggcacatacagcattcccagcagcttgaccaggggatggaggctgggatccattacgtcgaggctgtcttttccatgggtcctgtaacgcctgcccatgcaggagcctacagatgctgtggttgtttcagtcactcccgctatgagtggtcggctcccagtgaccccctggacattgtgatcacaggaaaatacaaaaagccttctctctccacccaggtggaccccatgatgaggctgggagagaagttgaccctcttctgcagctctgaaatctcatttgaccagtaccatctgttcagacacggggttgctcatggacagtggctcagtggagggcagagacacagggaagcattccaggccaacttttctgtgggccgtgcaacgccagtccctggcgggacctatagatgctatggttccttcaatgactctccctatgagtggtcagcccccagtgacccgctgcaactttacaccgacaaaactcacacatgcccaccgtgcccagcacctgaactcctggggggaccgtcagtcttcctcttccccccaaaacccaaggacaccctcatgatctcccggacccctgaggtcacatgcgtggtggtggacgtgagccacgaagaccctgaggtcaagttcaactggtacgtggacggcgtggaggtgcataatgccaagacaaagccgcgggaggagcagtacaacagcacgtaccgtgtggtcagcgtcctcaccgtcctgcaccaggactggctgaatggcaaggagtacaagtgcaaggtctccaacaaagccctcccagcccccatcgagaaaaccatctccaaagccaaagggcagccccgagaaccacaggtgtacaccctgcccccatcccgggaggagatgaccaagaaccaggtcagcctgacctgcctggtcaaaggcttctatcccagcgacatcgccgtggagtgggagagcaatgggcagccggagaacaactacaagaccacgcctcccgtgctggactccgacggctccttcttcctctacagcaagctcaccgtggacaagagcaggtggcagcaggggaacgtcttctcatgctccgtgatgcacgaggctctgcacaaccactacacgcagaagagcctctccctgtctccgggtaaatga

SEQ ID NO: 29 - DNA, 1374 bp, synthetic construct
  source 1..1374: mol_type = other DNA
atggcccccaaactcatcaccgtcctgtgtctgggattctgcctgaaccagaagatctgcccacatgcgggtgctcaggacaagttctccctgtcagcctggccgagccctgtggttcccctaggaggacgtgtgactctctcctgtcattcccatcttcggtttgtcatatggacaatattccaaacaactgggacccgaagccatgagttgcacactggcctttccaacaacatcaccatcagccctgtgaccccagaacacgcagggacctacagatgtgttggaatttacaagcacgcctcaaagtggtcagctgagagcaactccctgaagatcatcgtcacaggcttgttcacaaaaccctccatctcagcgcacccaagctccctggtgcatgcaggagccagggtgagcctgcgctgtcactcagaactggcctttgatgaatttatcttatacaaagaggggcacatacagcattcccagcagcttgaccaggggatggaggctgggatccattacgtcgaggctgtcttttccatgggtcctgtaacgcctgcccatgcaggagcctacagatgctgtggttgtttcagtcactcccgctatgagtggtcggctcccagtgaccccctggacattgtgatcacaggaaaatacaaaaagccttctctctccacccaggtggaccccatgatgaggctgggagagaagttgaccctcttctgcagctctgaaatctcatttgaccagtaccatctgttcagacacggggttgctcatggacagtggctcagtggagggcagagacacagggaagcattccaggccaacttttctgtgggccgtgcaacgccagtccctggcgggacctatagatgctatggttccttcaatgactctccctatgagtggtcagcccccagtgacccgctgcaactttacaccacaggaaacactaagagtactcctctgtcattcacagaatccacccctgaatctgacacacctcgccctcaaggacagtccagcaacctgcatatgctcactggactctcagtagccatcatctccattggcgtttgcctctctgcttttattggtttctggtgttacataaaatatcacaccaccatggcaaacacagagcccacggaaggccaacggacggatgaagaggagcctgcagcagaagagacacaggagatcatatatgcccagttaaaccaccaggccctctcacagacaggattccctcctgcctcccagtgtccccactacctctcggaggatcctagtatctacatcactgtccaccaagcccaggctgaggccagagctgcccccagtctttggcacaaagggcattaa

SEQ ID NO: 30 - DNA, 1629 bp, synthetic construct
  source 1..1629: mol_type = other DNA
atggcccccaaactcatcaccgtcctgtgtctgggattctgcctgaaccagaagatctgcccacatgcgggtgattacaaggatgacgatgacaaggctcaggacaagttctccctgtcagcctggccgagccctgtggttcccctaggaggacgtgtgactctctcctgtcattcccatcttcgatttgtcatatggacaatattccaaacaactgggacccgaagccatgagttgcacactggcctttccaacaacatcaccatcagccctgtgaccccagaacacgcagggacctacagatgtgttggaatttacaagcacgcctcaaagtggtcagctgagagcaactccctgaagatcatcgtcacaggcttgttcacaaaaccctccatctcagcgcacccaagctccctggtgcatgcaggagccagggtgagcctgcgctgtcactcagaactggcctttgatgaatttatcttatacaaagaggggcacatacagcattcccagcagcttgaccaggggatggaggctgggatccattacgtcgaggctgtcttttccatgggtcctgtaacgcctgcccatgcaggagcctacagatgctgtggttgtttcagtcactcccgctatgagtggtcggctcccagtgaccccctggacattgtgatcacaggaaaatacaaaaagccttctctctccacccaggtggaccccatgatgaggctgggagagaagttgaccctcttctgcagctctgaaatctcatttgaccagtaccatctgttcagacacggggttgctcatggacagtggctcagtggagggcagagacacagggaagcattccaggccaacttttctgtgggccgtgcaacgccagtccctggcgggacctatagatgctatggttccttcaatgactctccctatgagtggtcagcccccagtgacccgctgcaactttacaccacaggaaacactaagagtactcctctgtcattcacagaatccacccctgaatctgacacacctcgccctcaaggacagtccagcaacctgcatatgctcactctggtggtggttggtggagtcctggcttgctatagcttgctagtaacagtggcctttattattttctgggtgaggagtaagaggagcaggctcctgcacagtgactacatgaacatgactcccaggcggcccggacccacccgcaagcattaccagccctatgccccaccacgcgacttcgcagcctatcgctccgctagcctgagagtgaagttcagcaggagcgcagacgcccccgcgtaccagcagggccagaaccagctctataacgagctcaatctaggacgaagagaggagtacgatgttttggacaagagacgtggccgggaccctgagatggggggaaagccgcagagaaggaagaaccctcaggaaggcctgtacaatgaactgcagaaagataagatggcggaggcctacagtgagattgggatgaaaggcgagcgccggaggggcaaggggcacgatggcctttaccagggtctcagtacagccaccaaggacacctacgacgcccttcacatgcaggccctgccccctcgcgctagctga

SEQ ID NO: 31 - protein, 393 aa, synthetic construct
MAPKLITVLCLGFCLNQKICPHAGAQDKFSLSAWPSPVVPLGGRVTLSCHSHLRFVIWTIFQTTGTRSHELHTGLSNNITISPVTPEHAGTYRCVGIYKHASKWSAESNSLKIIVTGLFTKPSISAHPSSLVHAGARVSLRCHSELAFDEFILYKEGHIQHSQQLDQGMEAGIHYVEAVFSMGPVTPAHAGAYRCCGCFSHSRYEWSAPSDPLDIVITGKYKKPSLSTQVDPMMRLGEKLTLFCSSEISFDQYHLFRHGVAHGQWLSGGQRHREAFQANFSVGRATPVPGGTYRCYGSFNDSPYEWSAPSDPLQLYTTGNTKSTPLSFTESTPESDTPRPQGQSSNLHMLTILIGTSVVKIPFTILLFFLLHRWCSNKKKCCCNGPRACREQK

SEQ ID NO: 32 - DNA, 1182 bp, synthetic construct
  source 1..1182: mol_type = other DNA
atggcccccaaactcatcaccgtcctgtgtctgggattctgcctgaaccagaagatctgcccacatgcgggtgctcaggacaagttctccctgtcagcctggccgagccctgtggttcccctaggaggacgtgtgactctctcctgtcattcccatcttcggtttgtcatatggacaatattccaaacaactgggacccgaagccatgagttgcacactggcctttccaacaacatcaccatcagccctgtgaccccagaacacgcagggacctacagatgtgttggaatttacaagcacgcctcaaagtggtcagctgagagcaactccctgaagatcatcgtcacaggcttgttcacaaaaccctccatctcagcgcacccaagctccctggtgcatgcaggagccagggtgagcctgcgctgtcactcagaactggcctttgatgaatttatcttatacaaagaggggcacatacagcattcccagcagcttgaccaggggatggaggctgggatccattacgtcgaggctgtcttttccatgggtcctgtaacgcctgcccatgcaggagcctacagatgctgtggttgtttcagtcactcccgctatgagtggtcggctcccagtgaccccctggacattgtgatcacaggaaaatacaaaaagccttctctctccacccaggtggaccccatgatgaggctgggagagaagttgaccctcttctgcagctctgaaatctcatttgaccagtaccatctgttcagacacggggttgctcatggacagtggctcagtggagggcagagacacagggaagcattccaggccaacttttctgtgggccgtgcaacgccagtccctggcgggacctatagatgctatggttccttcaatgactctccctatgagtggtcagcccccagtgacccgctgcaactttacaccacaggaaacactaagagtactcctctgtcattcacagaatccacccctgaatctgacacacctcgccctcaaggacagtccagcaacctgcatatgctcactattctgattgggacctcagtggtcaaaatccctttcaccatcctcctcttctttctccttcatcgctggtgctccaacaaaaaaaaatgctgctgtaatggaccaagagcctgcagggaacagaagtga

SEQ ID NO: 33 - protein, 434 aa, Pan troglodytes
GAQDKFSLSAWPSPVVPLGGRVTLSCHSHLRFVIWTIFQTTGTRSHQLHTGLSNNITISPVTPGRAGTYRCVGIYKHTSKWSAESNSLKIIVTGLFTKPSISAHPSPLVHAGARVSLRCHSELAFDEFILYKEGHIQHSQQLDQGMEAGIHYVEAVFSVGPVTPAHAGAYRCCGCFSHSRYEWSAPSDPLDIVITGKYKKPSLSTQVDPMMRLGEKLTLFCSSEISFDQYHLFRDGVAHGQWLSGGQRHRGAFQANFSVGRSMPVPGGTYRCYGSFNDSPYEWSAPSDPLQLYATGNTKITPLSFTESTPESDTHRPQGQSSNLHMLTGLSVAIISIGVCLSAFIGFWCYIKYHTTMANTEPTEGQRTDEEEPAAEETQEIIYAQLNHQALSQTGFPPASQCPHYLSEEPSIYITVHQAQAEARAAPSLWHKGH

SEQ ID NO: 34 - protein, 434 aa, Gorilla gorilla
GAQDKFSLSAWPSPVVPLGGRVTLSCHSHLRFVIWTIFQTTGTRSHELHTGLSNNITISPVTPGHAGTYRCAGIYKHTSKWSAESNSLKIIVTGLFTKPSISAHPSSLVHAGARVSLRCHSELAFDEFILYKEGHIQHSQQLDQGMEAGIHYVEAVFSMGPITPAHAGAYRCCGCFSHSRYEWSAPSDSLDIVITGKYKKPSLSTQVGPMMRLGEKLTLFCSSEISFDQYHLFRDGVAHGQWLSGGQRHRGAFQANFSVGPAMPVPGGTYRCYGSFNDSPYEWSAPSDPLQLYATGNTKSTPLSFTESTPESDTHHPQGQSSNLHMLTGLSVAIISIGICLSAFIGFWCYIKYHTTMANTEPMEGQRTDEEEPAVEETQEIIYAQLNHQALSQTGFPPASQCPHYLSEEPSIYITVHQAQAEARAAPSLWHKRH

SEQ ID NO: 35 - protein, 434 aa, Pongo abelii
GAQDKFSLSAWPSPVVPLGGRVTLSCHSRLRFVVWTIFQTTGTRSRELHIGLSNNITISPVTPGHAGTYKCVGIYKHTSKWSAESNSLKIIVTGLFTKPAISAHPSSLVHAGTRVSLRCHSELAFDEFILYKEGRIQYSQQLDQGMEAGIHYVEAVFSMGPVTPAHAGAYRCCGCFSHSSYEWSAPSDPLDIVITGKYKKPSLSTQVDPMIRLGEKLTFFCSSEISFDWYHLLRDGVAHGQWLSGGQRHSGAFQANFSVGPATPVPGGTYRCYGSFNDSPYEWSAPSDPLHLYVTGNTKSTPLSLMESTHESDTHHPQGQSSNLNILIGLSVAIISIGVCLSAFIGFWCYIKYYTTMANTEPMEGQRTDEEEPAAEETQKIIYAQLNHQALSQTGFTPASPCPHYLSEDPSIYVTVHQAQAEARAAPSLWHKGH

SEQ ID NO: 36 - protein, 99 aa, Pan paniscus
GKYKKPSLSTQVDPMMRLGEKLTLFCSSEISFDQYRLFRDGVAHGQWLSGGQRHRGAFQANFSVGRSMPVPGGTYRCYGSFNDSPYEWSAPSDPLQLYA

SEQ ID NO: 37 - protein, 325 aa, Pan paniscus
GAQDKFSLSAWPSPVVPLGGRVTLSCHSHLRFVIWTIFQTTGTRSHQLHIGLSNNITISPVTPGHAGTYRCVGIYKHTSKWSAESNSLKIIVTGLFTKPCISAHPSPLVHAGARVSLRCHSELAFDEFILYKEGHIQHSQQLDQGMEAGIHYVEAVFSVGPVTPAHAGAYRCCGCFSHSRYEWSAPSDPLDIVITGKYKKPSLSTQVDPMMRLGEKLTLFCSSEISFDQYRLFRDGVAHGQWLSGGQRHRGAFQANFSVGRSMPVPGGTYRCYGSFNDSPYEWSAPSDPLQLYATGNTKITPLSFTESTPESDTHRPQGQSSNLH

SEQ ID NO: 38 - protein, 434 aa, Pan paniscus
GAQDKFSLSAWPSPVVPLGGRVTLSCHSHLRFVIWTIFQTTGTRSHQLHIGLSNNITISPVTPGHAGTYRCVGIYKHTSKWSAESNSLKIIVTGLFTKPCISAHPSPLVHAGARVSLRCHSELAFDEFILYKEGHIQHSQQLDQGMEAGIHYVEAVFSVGPVTPAHAGAYRCCGCFSHSRYEWSAPSDPLDIVITGKYKKPSLSTQVDPMMRLGEKLTLFCSSEISFDQYRLFRDGVAHGQWLSGGQRHRGAFQANFSVGRSMPVPGGTYRCYGSFNDSPYEWSAPSDPLQLYATGNTKITPLSFTESTPESDTHRPQGQSSNLHMLTGLSVAIISIGVCLSAFIGFWCYIKYHTTMANTEPTEGQRTDEEEPAAEETQEIIYAQLNHQALSQTGFPPVSQCPHYLSEEPSIYITVHQAQAEARAAPSLWHKGH

SEQ ID NO: 39 - protein, 13 aa, Pongo abelii
EWSAPSDPLHLYV

SEQ ID NO: 40 - DNA, 53 bp, Homo sapiens
  source 1..53: mol_type = genomic DNA
  variation 32..33: note = 7 bp deletion in exon 5
gatgctatggttccttcaatgactctccctataagcccccagtgacccgctgc

SEQ ID NO: 41 - DNA, 60 bp, Pan troglodytes
  source 1..60: mol_type = genomic DNA
gatgctatggttccttcaatgactctccctatgagtggtcagcccccagtgacccgctgc

SEQ ID NO: 42 - DNA, 60 bp, Gorilla gorilla
  source 1..60: mol_type = genomic DNA
gatgctacggctccttcaatgactctccctatgagtggtcagcccccagtgacccgctgc

SEQ ID NO: 43 - DNA, 60 bp, Pongo abelii
  source 1..60: mol_type = genomic DNA
gatgctatggttctttcaatgactctccctatgagtggtcagcccccagtgacccactac

SEQ ID NO: 44 - DNA, 60 bp, Nomascus leucogenys
  source 1..60: mol_type = genomic DNA
gatgctatggttctttcaatgactctccctatgagtggtcagcccccagtgacccactgc

SEQ ID NO: 45 - DNA, 60 bp, Macaca leonina; identical to SEQ ID NO: 44
  source 1..60: mol_type = genomic DNA

SEQ ID NO: 46 - DNA, 60 bp, Papio anubis; identical to SEQ ID NO: 44
  source 1..60: mol_type = genomic DNA

SEQ ID NO: 47 - DNA, 60 bp, Colobus angolensis; identical to SEQ ID NO: 44
  source 1..60: mol_type = genomic DNA

SEQ ID NO: 48 - DNA, 60 bp, Theropithecus gelada
  source 1..60: mol_type = genomic DNA
gatgctatgattctttcaatgactctccctatgagtggtcagctcccagtgacccactgc

SEQ ID NO: 49 - DNA, 60 bp, Macaca mulatta
  source 1..60: mol_type = genomic DNA
gatgctatggttctttcaatgactctccctatgagtggtcagcccccagtgaccccctgc

SEQ ID NO: 50 - DNA, 60 bp, Macaca fascicularis; identical to SEQ ID NO: 49
  source 1..60: mol_type = genomic DNA

SEQ ID NO: 51 - DNA, 60 bp, Macaca nemestrina; identical to SEQ ID NO: 49
  source 1..60: mol_type = genomic DNA

SEQ ID NO: 52 - DNA, 60 bp, Cercocebus atys
  source 1..60: mol_type = genomic DNA
gatgctatggttctttcaatgactctccctatgtgtggtcagcccccagtgaccccctgc

SEQ ID NO: 53 - DNA, 60 bp, Rhinopithecus roxellana
  source 1..60: mol_type = genomic DNA
gatgctatggttctttcaatgactctccctatgtgtggtcagcccccagtgacccactgc

SEQ ID NO: 54 - DNA, 60 bp, Rhinopithecus bieti; identical to SEQ ID NO: 53
  source 1..60: mol_type = genomic DNA

SEQ ID NO: 55 - DNA, 60 bp, Trachypithecus francoisi
  source 1..60: mol_type = genomic DNA
catgctatggttctttcaatgactctccctacgtgtggtcagcccccagtgacccactgc

SEQ ID NO: 56 - DNA, 60 bp, Callithrix jacchus
  source 1..60: mol_type = genomic DNA
gatgctacggttctttcaatgcctccccctatgagtggtcggcccccagtgagcccctgc

SEQ ID NO: 57 - DNA, 60 bp, Saimiri boliviensis
  source 1..60: mol_type = genomic DNA
gatgctacggttctttcaatgcctccccgtatgagtggtcagcccccagtgagcccctgc

SEQ ID NO: 58 - DNA, 60 bp, Carlito syrichta
  source 1..60: mol_type = genomic DNA
gatgctatggttctttcagtcactcccgctatgagtggccagcccctagtgaccccctgg

SEQ ID NO: 59 - DNA, 60 bp, Microcebus murinus
  source 1..60: mol_type = genomic DNA
gatgctacggctacttctatttctccccccataagtggtcatccccaagtgaccccctgc

SEQ ID NO: 60 - protein, 99 aa, Symphalangus syndactylus
GKYKKPSLSTHVDPMMKLGEKLTFFCSSEISFDWYHLFRDGVAHGQWLSGGQRCSGAFQANFSVGPATPVPGGTYRCYGSFNGSPYEWSAPSDPLHLYV

SEQ ID NO: 61 - protein, 324 aa, Symphalangus syndactylus
GAQFKLSLSAWPSPVVPLGGCVTLSCHPRLRFLVLTIVQTTGTRTRELHAGLSNITISPVTPGHAGTYKCVGIYKHTSKWSAESNSLKIIVTGVFTKPSIAAHPSSVVHAGARVSLRCHSELAFDEFVLYKDGHIQHSQQLEEGMEAGIHYVEAVFSVGPVTPAHAGAYRCCGCFSHSSYEWSAPSDPLDIVITGKYKKPSLSTHVDPMMKLGEKLTFFCSSEISFDWYHLFRDGVAHGQWLSGGQRCSGAFQANFSVGPATPVPGGTYRCYGSFNGSPYEWSAPSDPLHLYVTGNTKSTPLSFMESTPESDTHRPQGQSSNWN

SEQ ID NO: 62 - protein, 433 aa, Symphalangus syndactylus
GAQFKLSLSAWPSPVVPLGGCVTLSCHPRLRFLVLTIVQTTGTRTRELHAGLSNITISPVTPGHAGTYKCVGIYKHTSKWSAESNSLKIIVTGVFTKPSIAAHPSSVVHAGARVSLRCHSELAFDEFVLYKDGHIQHSQQLEEGMEAGIHYVEAVFSVGPVTPAHAGAYRCCGCFSHSSYEWSAPSDPLDIVITGKYKKPSLSTHVDPMMKLGEKLTFFCSSEISFDWYHLFRDGVAHGQWLSGGQRCSGAFQANFSVGPATPVPGGTYRCYGSFNGSPYEWSAPSDPLHLYVTGNTKSTPLSFMESTPESDTHRPQGQSSNWNVLIGLSVAIISTGVCLSAFIGFWCYIKYDTTMANTETMEGQRTDEEEPAAEETQEIMYAQLNHQALSQIGFTAASQCPHYLSEEPSIYITVHQVQAEDRAAPSLWHKGH